European Patent Specification EP 4 139 474 B1, published January 1, 2025. Title: Diagnostic Control Compositions. Applicant: University of the Witwatersrand, Johannesburg. The sequence listing filed with the application follows.

SEQUENCE LISTING (28 sequences)

SEQ ID NO: 1 - DNA, 474 bp, Mycobacterium bovis
gttaacactagttgattagctaagcagaaggccatcctgacggatggcctttttgcgtttaatactgtttaaacctctagaggtgtggtagccgatgccggtgttggcgccggtgaccacaacgacgcgcccgctttgatcggggacgtctgcggccgaccatttacgggtcttgttgtcgttggcggtcatgggccgaacatactcacccggatcggagggccgaggacaaggtcgaacgaggggcatgacccggtgcggggcttcttgcactcggcataggcgagtgctaagaataacgttggcactcgcgaccggtgagtgctaggtcgggacggtgaggccaggcccgtcgtcgcagcgagtggcagcgaggacaacttgagccgtccgtcgcgggcactgcgcccggccagcgtaagtagcggggttgccgtcacccggtgacccccgtttcatccccgatccgcatgc

SEQ ID NO: 2 - DNA, 209 bp, SARS-CoV-2
ctcttattgtaacagctttaagggccaattctgctgtcaaattacagaataatgagcttagtcctgttgcactacgacagatgtcttgtgctgccggtactacacaaactgcttgcactgatgacaatgcgttagcttactacaacacaacaaagggaggtaggtttgtacttgcactgttatccgatttacaggatttgaaatgggct

SEQ ID NO: 3 - DNA, 207 bp, SARS-CoV-2
gaaatgctggtattgttggtgtactgacattagataatcaagatctcaatggtaactggtatgatttcggtgatttcatacaaaccacgccaggtagtggagttcctgttgtagattcttattattcattgttaatgcctatattaaccttgaccagggctttaactgcagagtcacatgttgacactgacttaacaaagccttaca

SEQ ID NO: 4 - DNA, 1100 bp, SARS-CoV-2
tttagatttcatctaaacgaacaaactaaaatgtctgataatggaccccaaaatcagcgaaatgcaccccgcattacgtttggtggaccctcagattcaactggcagtaaccagaatggagaacgcagtggggcgcgatcaaaacaacgtcggccccaaggtttacccaataatactgcgtcttggttcaccgctctcactcaacatggcaaggaagaccttaaattccctcgaggacaaggcgttccaattaacaccaatagcagtccagatgaccaaattggctactaccgaagagctaccagacgaattcgtggtggtgacggtaaaatgaaagatctcagtccaagatggtatttctactacctaggaactgggccagaagctggacttccctatggtgctaacaaagacggcatcatatgggttgcaactgagggagccttgaatacaccaaaagatcacattggcacccgcaatcctgctaacaatgctgcaatcgtgctacaacttcctcaaggaacaacattgccaaaaggcttctacgcagaagggagcagaggcggcagtcaagcctcttctcgttcctcatcacgtagtcgcaacagttcaagaaattcaactccaggcagcagtaggggaacttctcctgctagaatggctggcaatggcggtgatgctgctcttgctttgctgctgcttgacagattgaaccagcttgagagcaaaatgtctggtaaaggccaacaacaacaaggccaaactgtcactaagaaatctgctgctgaggcttctaagaagcctcggcaaaaacgtactgccactaaagcatacaatgtaacacaagctttcggcagacgtggtccagaacaaacccaaggaaattttggggaccaggaactaatcagacaaggaactgattacaaacattggccgcaaattgcacaatttgcccccagcgcttcagcgttcttcggaatgtcgcgcattggcatggaagtcacaccttcgggaacgtggttgacctacacaggtgccatcaaattggatgacaaagatccaaatttcaaagatcaagtcattttgctgaataagcatat

SEQ ID NO: 5 - DNA, 222 bp, SARS-CoV-2
tcattcgtttcggaagagacaggtacgttaatagttaatagcgtacttctttttcttgctttcgtggtattcttgctagttacactagccatccttactgcgcttcgattgtgtgcgtactgctgcaatattgttaacgtgagtcttgtaaaaccttctttttacgtttactctcgtgttaaaaatctgaattcttctagagttcctgatcttctggtctaa

SEQ ID NO: 6 - DNA, 328 bp, SARS-CoV-2
aaattgattgccaaccaatttaatagtgctattggcaaaattcaagactcactttcttccacagcaagtgcacttggaaaacttcaagatgtggtcaaccaaaatgcacaagctttaaacacgcttgttaaacaacttagctccaattttggtgcaatttcaagtgttttaaatgatatcctttcacgtcttgacaaagttgaggctgaagtgcaaattgataggttgatcacaggcagacttcaaagtttgcagacatatgtgactcaacaattaattagagctgcagaaatcagagcttctgctaatcttgctgctactaaaatgt

SEQ ID NO: 7 - DNA, 400 bp, SARS-CoV-2
acttgaacagccctatgtgttcatcaaacgttcggatgctcgaactgcacctcatggtcatgttatggttgagctggtagcagaactcgaaggcattcagtacggtcgtagtggtgagacacttggtgtccttgtccctcatgtgggcgaaataccagtggcttaccgcaaggttcttcttcgtaagaacggtaataaaggagctggtggccatagttacggcgccgatctaaagtcatttgacttaggcgacgagcttggcactgatccttatgaagattttcaagaaaactggaacactaaacatagcagtggtgttacccgtgaactcatgcgtgagcttaacggaggggcatacactcgctatgtcgataacaacttctgtggccctgatggctac

SEQ ID NO: 8 - DNA, 775 bp, Artemia salina
aggaaggaatgtacatatggcgaccgagggcgcgcgcaacatcggccagtcggccccggagggcaaggtgcagatggactgcccgtcgcgccacaacttcgacccggagtgcgagaaggcgtttgtggagcacatccaccttgagctggcctcgtcgtaccacgcatggtcgatgtgggccttctacgcccgcgactgcaaggccgccgtgggcatgacccgcctgtgcgagtgggcctcgcacgtctcggcccagcgcgcccgccgcatggccgcctacgtgctgacccgcggcggccacgtggactacaaggagatcccggccccgaagaagcagggctgggacaacttcgaggacgccttctcgcactgcgtggcgaacaagaagcgcatcctgacctcgctccagtcgctgtaccagtgctgccagtcgaaggacgcccactgctcgaacttcatccagaccgacatgatggacgaggtgatcgcgtggaacaagtttctgtcggactgcctgtcgaacctgcactgcatcggctcgcagggcatgggaccgtgggtgttcgaccgctggctggcccgcatcgtgatgtcgaagttcaagcacccgaagatcccgtcgctctcgacctcggacctagagtcgaacatcccgaacgagctgttcgacgccgagggcgacatggtgcgcgccatcaagaagctggactacaaggaccatgacggtgactataaagatcacgatatagattacaaggatgacgatgacaagtga

SEQ ID NO: 9 - DNA, 888 bp, Bacteriophage GBSV1
atgcataccatctaccgcatcgagaagaaggagaactacgtggtgctggacaagggcttcctgcacgaccgcgagctgtcgtggcaggctaagggcctgctggccttcatgctgtcgatgccgaacgactgggtgttcaacatgaaggacctccagaaccgctcgaagaacggtcgcgacgccacctaccgcattatgaaggagctgatcgaggccggctacgtgacccgcgtggagaaccgcgacggcggcaagttcggcaaggtggagtacgtggtccacgaggtgaagcagtcgccgcacaccgagtcgccggacaccgtgccgccctgcaccgagaacccgtaccccggcaacccgtaccccggcaacccgtacccggagaacccgccgctgctgaacaacaacaacaccaactacaagaacaccaacaacgacgacgacaacaaggaccgcccgaagaccaactcgctgaacgcctttcgcttctacgaggagaacttccagccgaccctgtcgtcggtggacatcgagatcctgaactactggctggaccgcttcccggaggagatcgtgctgtgcgccatgcggaaggccctagagcagaacgtgcgctcgatcaagtacatcgaccgcatccttgccaactgggagatgcagaaggtgcagacccttgaggacgtggcccgcctcgaccgccagtacgagctggagaagcaggcccgccagaagcgcggcggcgtggtgaacggctcggtccaccagcaccgcggctcggacggtcgctcgacgaaggaggacgagcgcatctcgcactacgagccgggcaagtgggacgacgtggacatctcgctggacggcctgctgcaccatcaccaccatcactga

SEQ ID NO: 10 - DNA, 1005 bp, Escherichia coli
gatctgcattaatgaatcggccaacgcgcggggagaggcggtttgcgtattgggcgctcttccgcttcctcgctcactgactcgctgcgctcggtcgttcggctgcggcgagcggtatcagctcactcaaaggcggtaatacggttatccacagaatcaggggataacgcaggaaagaacatgtgagcaaaaggccagcaaaaggccaggaaccgtaaaaaggccgcgttgctggcgtttttccataggctccgcccccctgacgagcatcacaaaaatcgacgctcaagtcagaggtggcgaaacccgacaggactataaagataccaggcgtttccccctggaagctccctcgtgcgctctcctgttccgaccctgccgcttaccggatacctgtccgcctttctcccttcgggaagcgtggcgctttctcatagctcacgctgtaggtatctcagttcggtgtaggtcgttcgctccaagctgggctgtgtgcacgaaccccccgttcagcccgaccgctgcgccttatccggtaactatcgtcttgagtccaacccggtaagacacgacttatcgccactggcagcagccactggtaacaggattagcagagcgaggtatgtaggcggtgctacagagttcttgaagtggtggcctaactacggctacactagaagaacagtatttggtatctgcgctctgctgaagccagttaccttcggaaaaagagttggtagctcttgatccggcaaacaaaccaccgctggtagcggtggtttttttgtttgcaagcagcagattacgcgcagaaaaaaaggatctcaagaagatcctttgatcttttctacggggtctgacgctcagtggaacgaaaactcacgttaagggattttggtcatgagattatcaaaaaggatcttcacctagatccttttaaattaaaaatgaagttttaaatcaagcccaatctgaataatgttacaaccaattaaccaattctga

SEQ ID NO: 11 - DNA, 810 bp, Artificial Sequence
  Kanamycin resistance cassette
atgagccatattcaacgggaaacgtcgaggccgcgattaaattccaacatggatgctgatttatatgggtataaatgggctcgcgataatgtcgggcaatcaggtgcgacaatctatcgcttgtatgggaagcccgatgcgccagagttgtttctgaaacatggcaaaggtagcgttgccaatgatgttacagatgagatggtcagactaaactggctgacggaatttatgcctcttccgaccatcaagcattttatccgtactcctgatgatgcatggttactcaccactgcgatccccggaaaaacagcattccaggtattagaagaatatcctgattcaggtgaaaatattgttgatgcgctggcagtgttcctgcgccggttgcattcgattcctgtttgtaattgtccttttaacagcgatcgcgtatttcgtctcgctcaggcgcaatcacgaatgaataacggtttggttgatgcgagtgattttgatgacgagcgtaatggctggcctgttgaacaagtctggaaagaaatgcataaacttttgccattctcaccggattcagtcgtcactcatggtgatttctcacttgataaccttatttttgacgaggggaaattaataggttgtattgatgttggacgagtcggaatcgcagaccgataccaggatcttgccatcctatggaactgcctcggtgagttttctccttcattacagaaacggctttttcaaaaatatggtattgataatcctgatatgaataaattgcagtttcatttgatgctcgatgagtttttctaa

SEQ ID NO: 12 - DNA, 2369 bp, pYUB12
ggggcctgtaacggcacaacgaaccgtgcaacgagagtggccacggatgccaccacaagcactacaacggagttcgccacgtacatcaccacaaccaccgattctggcggtgagctccacgatattcagcggaaatggcttggtatcgaccaagattcgtagaaccccgtctcgtctggctggtattcaaaacggacgcaacgaaacacgcaacgagacaggcatggcccaaaccagaaaactagcgtctaccaggacttttacctgtccgacccgttgcaacggaaccccccacggaacccccgcgacacccgctccccaattgcgttagaacagcggtggattgtcggcttcgttgtgggccttttgagccgcttcctgttctgccgcacgctctttcctcgcccgatagccgagtcgcttaacggtgtccagatgcagcccgaaatgtttggccgtttgcggccaagagtggccctcgtcgtcgtgataggcgcggatgcgttcgcggcgtgcagcctgctcggcgagccactcgctgcgttcctgcgccacgagccggacgacgtggcgttcggatagtccggtgattcgagcgccttcggcggcggtcacgcgccgctttttgcggacagtcggctgccggttgtagccgtcgctgtagccgtcgctgtagccgtcgctcatagcaatgcctccatggctgacgcggactttgcgcgccgcgcaactgtgctcgccgccgtgcgcgctgctgcgcccttccgcgagatggccgactggcgcgcactgagtgtggcctcgtagaccacgatcccgtccgcccaaatgcgcgacttggttgtgatccaacgccaaatgctgttggcgatggcgcggacctcgctgtccggtagcggtccgggacacacgtcgttgcacgggaattcggcgtttcgcgcgtggcactcggcatagatcgcgcggccgagtccgtccacgttccgggtcggcaggtagatccgcatgagggcgggacgataggcccacaacctgacggaatcgaacagtgcgcaattccgccctagcggcgtcggagccgctttgtacgtggtctgctgacgccagcgcggcggtggcatgttcgcgccgagctcggcctcgatgtggctgagtgtgtagagatctgagtggagccattccgtttcccaggcgatgtggccggggtttttggtcatgaggcctgagtaactgcggtcgccgtcgacggcgcgccgaaggccttcggcgcacgccgccatgtatgcgagcggcttacgccgcgcgtattcggtgcgtggaacaggggcgttgagtgcccacactgcgtgtgcgtggccgttggcgcgattgcccacgatcgcgttgggcagcggatgggacccccgggcgctgagcgctcggagcgctgcgtctggatggtctacgtccacgaccagcaggtttgccagcgctgttgggttcgcctcgatgtaccggcggcctagggccgacgcgcggctttggcggtagatcccctcgagcagatcgtcgcttgccagcggccagtacggcagccagagctgctcaaattcgtcggcgacgtggctcacgcttggtagtagaccacgattaatcaccggtgtatggtccgacacgagctccaagtcagatatttcgctgaggggccaccccacaactgcacactcccccgctctcccgtcgagccctgatgatgaaacaccagcgacagccgagcacccccaaccacctgtaccaaccaggaggaacacatgcgtcgtttcgaggacgtttccgggccgctaagagccgctgtggcggccgtacacgccgccttagacccgttagaccccctgccgcctgaatgcgcgggtacgagccacacagcacccgaacttacggagctggtgggctcacctggctttatggcgtacgaatcggctgtgtgcgacctgttgggcgaggtgagatacgcgctactcacgctggcaagggcgacacagccgccccaccgagcccgcacggccgcgcgcggtgtcaacaaccgggtgagtcgtgcacaccagcaggtgttcgaggcttggctcgaagtgcaggacatcgtggcgaacgccgcccgatgagccgcgccttacgctggctgccagccgttcgcgggctggttggtgcagcgcgtcgagcggttagaggccctgcggtgttccaccaccgcaggcctcgccctttttaaggctgaatttgcttgtctccgaatccaactggcttgtccaagggtgtatctacgcttagtccaaagttcaaacgaggggattacacatgaccaacttcgataacgttctcggctcgatctg

SEQ ID NO: 13 - DNA, 56 bp, Artificial Sequence
  Theophylline riboswitch
ggtgataccagcatcgtcttgatgccctggcagcaccctgctaaggaggcaacaag

SEQ ID NO: 14 - DNA, 4022 bp, Artificial Sequence
  DNA cassette for targets RdRp1, RdRp2, N protein and E protein
gttaacactagttgattagctaagcagaaggccatcctgacggatggcctttttgcgtttaatactgtttaaacctctagaggtgtggtagccgatgccggtgttggcgccggtgaccacaacgacgcgcccgctttgatcggggacgtctgcggccgaccatttacgggtcttgttgtcgttggcggtcatgggccgaacatactcacccggatcggagggccgaggacaaggtcgaacgaggggcatgacccggtgcggggcttcttgcactcggcataggcgagtgctaagaataacgttggcactcgcgaccggtgagtgctaggtcgggacggtgaggccaggcccgtcgtcgcagcgagtggcagcgaggacaacttgagccgtccgtcgcgggcactgcgcccggccagcgtaagtagcggggttgccgtcacccggtgacccccgtttcatccccgatccgcatgcggatccctgcagagtactctcttattgtaacagctttaagggccaattctgctgtcaaattacagaataatgagcttagtcctgttgcactacgacagatgtcttgtgctgccggtactacacaaactgcttgcactgatgacaatgcgttagcttactacaacacaacaaagggaggtaggtttgtacttgcactgttatccgatttacaggatttgaaatgggctagtactcagctggaaatgctggtattgttggtgtactgacattagataatcaagatctcaatggtaactggtatgatttcggtgatttcatacaaaccacgccaggtagtggagttcctgttgtagattcttattattcattgttaatgcctatattaaccttgaccagggctttaactgcagagtcacatgttgacactgacttaacaaagccttacacagctggatatctttagatttcatctaaacgaacaaactaaaatgtctgataatggaccccaaaatcagcgaaatgcaccccgcattacgtttggtggaccctcagattcaactggcagtaaccagaatggagaacgcagtggggcgcgatcaaaacaacgtcggccccaaggtttacccaataatactgcgtcttggttcaccgctctcactcaacatggcaaggaagaccttaaattccctcgaggacaaggcgttccaattaacaccaatagcagtccagatgaccaaattggctactaccgaagagctaccagacgaattcgtggtggtgacggtaaaatgaaagatctcagtccaagatggtatttctactacctaggaactgggccagaagctggacttccctatggtgctaacaaagacggcatcatatgggttgcaactgagggagccttgaatacaccaaaagatcacattggcacccgcaatcctgctaacaatgctgcaatcgtgctacaacttcctcaaggaacaacattgccaaaaggcttctacgcagaagggagcagaggcggcagtcaagcctcttctcgttcctcatcacgtagtcgcaacagttcaagaaattcaactccaggcagcagtaggggaacttctcctgctagaatggctggcaatggcggtgatgctgctcttgctttgctgctgcttgacagattgaaccagcttgagagcaaaatgtctggtaaaggccaacaacaacaaggccaaactgtcactaagaaatctgctgctgaggcttctaagaagcctcggcaaaaacgtactgccactaaagcatacaatgtaacacaagctttcggcagacgtggtccagaacaaacccaaggaaattttggggaccaggaactaatcagacaaggaactgattacaaacattggccgcaaattgcacaatttgcccccagcgcttcagcgttcttcggaatgtcgcgcattggcatggaagtcacaccttcgggaacgtggttgacctacacaggtgccatcaaattggatgacaaagatccaaatttcaaagatcaagtcattttgctgaataagcatatgatatctacgtactcattcgtttcggaagagacaggtacgttaatagttaatagcgtacttctttttcttgctttcgtggtattcttgctagttacactagccatccttactgcgcttcgattgtgtgcgtactgctgcaatattgttaacgtgagtcttgtaaaaccttctttttacgtttactctcgtgttaaaaatctgaattcttctagagttcctgatcttctggtctaatacgtaaagcttaggaaggaatgtacatatggcgaccgagggcgcgcgcaacatcggccagtcggccccggagggcaaggtgcagatggactgcccgtcgcgccacaacttcgacccggagtgcgagaaggcgtttgtggagcacatccaccttgagctggcctcgtcgtaccacgcatggtcgatgtgggccttctacgcccgcgactgcaaggccgccgtgggcatgacccgcctgtgcgagtgggcctcgcacgtctcggcccagcgcgcccgccgcatggccgcctacgtgctgacccgcggcggccacgtggactacaaggagatcccggccccgaagaagcagggctgggacaacttcgaggacgccttctcgcactgcgtggcgaacaagaagcgcatcctgacctcgctccagtcgctgtaccagtgctgccagtcgaaggacgcccactgctcgaacttcatccagaccgacatgatggacgaggtgatcgcgtggaacaagtttctgtcggactgcctgtcgaacctgcactgcatcggctcgcagggcatgggaccgtgggtgttcgaccgctggctggcccgcatcgtgatgtcgaagttcaagcacccgaagatcccgtcgctctcgacctcggacctagagtcgaacatcccgaacgagctgttcgacgccgagggcgacatggtgcgcgccatcaagaagctggactacaaggaccatgacggtgactataaagatcacgatatagattacaaggatgacgatgacaagtgacttaagggtaccggtgataccagcatcgtcttgatgccctggcagcaccctgctaaggaggcaacaagatgcataccatctaccgcatcgagaagaaggagaactacgtggtgctggacaagggcttcctgcacgaccgcgagctgtcgtggcaggctaagggcctgctggccttcatgctgtcgatgccgaacgactgggtgttcaacatgaaggacctccagaaccgctcgaagaacggtcgcgacgccacctaccgcattatgaaggagctgatcgaggccggctacgtgacccgcgtggagaaccgcgacggcggcaagttcggcaaggtggagtacgtggtccacgaggtgaagcagtcgccgcacaccgagtcgccggacaccgtgccgccctgcaccgagaacccgtaccccggcaacccgtaccccggcaacccgtacccggagaacccgccgctgctgaacaacaacaacaccaactacaagaacaccaacaacgacgacgacaacaaggaccgcccgaagaccaactcgctgaacgcctttcgcttctacgaggagaacttccagccgaccctgtcgtcggtggacatcgagatcctgaactactggctggaccgcttcccggaggagatcgtgctgtgcgccatgcggaaggccctagagcagaacgtgcgctcgatcaagtacatcgaccgcatccttgccaactgggagatgcagaaggtgcagacccttgaggacgtggcccgcctcgaccgccagtacgagctggagaagcaggcccgccagaagcgcggcggcgtggtgaacggctcggtccaccagcaccgcggctcggacggtcgctcgacgaaggaggacgagcgcatctcgcactacgagccgggcaagtgggacgacgtggacatctcgctggacggcctgctgcaccatcaccaccatcactgaacgcgtatcgat

SEQ ID NO: 15 - DNA, 4770 bp, Artificial Sequence
  DNA cassette for targets Spike protein, ORF1ab 5' region, RdRp1, RdRp2, N protein and E protein
gttaacactagttgattagctaagcagaaggccatcctgacggatggcctttttgcgtttaatactgtttaaacctctagaggtgtggtagccgatgccggtgttggcgccggtgaccacaacgacgcgcccgctttgatcggggacgtctgcggccgaccatttacgggtcttgttgtcgttggcggtcatgggccgaacatactcacccggatcggagggccgaggacaaggtcgaacgaggggcatgacccggtgcggggcttcttgcactcggcataggcgagtgctaagaataacgttggcactcgcgaccggtgagtgctaggtcgggacggtgaggccaggcccgtcgtcgcagcgagtggcagcgaggacaacttgagccgtccgtcgcgggcactgcgcccggccagcgtaagtagcggggttgccgtcacccggtgacccccgtttcatccccgatccgcatgcggatctcgacacttgaacagccctatgtgttcatcaaacgttcggatgctcgaactgcacctcatggtcatgttatggttgagctggtagcagaactcgaaggcattcagtacggtcgtagtggtgagacacttggtgtccttgtccctcatgtgggcgaaataccagtggcttaccgcaaggttcttcttcgtaagaacggtaataaaggagctggtggccatagttacggcgccgatctaaagtcatttgacttaggcgacgagcttggcactgatccttatgaagattttcaagaaaactggaacactaaacatagcagtggtgttacccgtgaactcatgcgtgagcttaacggaggggcatacactcgctatgtcgataacaacttctgtggccctgatggctacaagcttaaattgattgccaaccaatttaatagtgctattggcaaaattcaagactcactttcttccacagcaagtgcacttggaaaacttcaagatgtggtcaaccaaaatgcacaagctttaaacacgcttgttaaacaacttagctccaattttggtgcaatttcaagtgttttaaatgatatcctttcacgtcttgacaaagttgaggctgaagtgcaaattgataggttgatcacaggcagacttcaaagtttgcagacatatgtgactcaacaattaattagagctgcagaaatcagagcttctgctaatcttgctgctactaaaatgtagatcgatccctgcagagtactctcttattgtaacagctttaagggccaattctgctgtcaaattacagaataatgagcttagtcctgttgcactacgacagatgtcttgtgctgccggtactacacaaactgcttgcactgatgacaatgcgttagcttactacaacacaacaaagggaggtaggtttgtacttgcactgttatccgatttacaggatttgaaatgggctagtactcagctggaaatgctggtattgttggtgtactgacattagataatcaagatctcaatggtaactggtatgatttcggtgatttcatacaaaccacgccaggtagtggagttcctgttgtagattcttattattcattgttaatgcctatattaaccttgaccagggctttaactgcagagtcacatgttgacactgacttaacaaagccttacacagctggatatctttagatttcatctaaacgaacaaactaaaatgtctgataatggaccccaaaatcagcgaaatgcaccccgcattacgtttggtggaccctcagattcaactggcagtaaccagaatggagaacgcagtggggcgcgatcaaaacaacgtcggccccaaggtttacccaataatactgcgtcttggttcaccgctctcactcaacatggcaaggaagaccttaaattccctcgaggacaaggcgttccaattaacaccaatagcagtccagatgaccaaattggctactaccgaagagctaccagacgaattcgtggtggtgacggtaaaatgaaagatctcagtccaagatggtatttctactacctaggaactgggccagaagctggacttccctatggtgctaacaaagacggcatcatatgggttgcaactgagggagccttgaatacaccaaaagatcacattggcacccgcaatcctgctaacaatgctgcaatcgtgctacaacttcctcaaggaacaacattgccaaaaggcttctacgcagaagggagcagaggcggcagtcaagcctcttctcgttcctcatcacgtagtcgcaacagttcaagaaattcaactccaggcagcagtaggggaacttctcctgctagaatggctggcaatggcggtgatgctgctcttgctttgctgctgcttgacagattgaaccagcttgagagcaaaatgtctggtaaaggccaacaacaacaaggccaaactgtcactaagaaatctgctgctgaggcttctaagaagcctcggcaaaaacgtactgccactaaagcatacaatgtaacacaagctttcggcagacgtggtccagaacaaacccaaggaaattttggggaccaggaactaatcagacaaggaactgattacaaacattggccgcaaattgcacaatttgcccccagcgcttcagcgttcttcggaatgtcgcgcattggcatggaagtcacaccttcgggaacgtggttgacctacacaggtgccatcaaattggatgacaaagatccaaatttcaaagatcaagtcattttgctgaataagcatatgatatctacgtactcattcgtttcggaagagacaggtacgttaatagttaatagcgtacttctttttcttgctttcgtggtattcttgctagttacactagccatccttactgcgcttcgattgtgtgcgtactgctgcaatattgttaacgtgagtcttgtaaaaccttctttttacgtttactctcgtgttaaaaatctgaattcttctagagttcctgatcttctggtctaatacgtaaagcttaggaaggaatgtacatatggcgaccgagggcgcgcgcaacatcggccagtcggccccggagggcaaggtgcagatggactgcccgtcgcgccacaacttcgacccggagtgcgagaaggcgtttgtggagcacatccaccttgagctggcctcgtcgtaccacgcatggtcgatgtgggccttctacgcccgcgactgcaaggccgccgtgggcatgacccgcctgtgcgagtgggcctcgcacgtctcggcccagcgcgcccgccgcatggccgcctacgtgctgacccgcggcggccacgtggactacaaggagatcccggccccgaagaagcagggctgggacaacttcgaggacgccttctcgcactgcgtggcgaacaagaagcgcatcctgacctcgctccagtcgctgtaccagtgctgccagtcgaaggacgcccactgctcgaacttcatccagaccgacatgatggacgaggtgatcgcgtggaacaagtttctgtcggactgcctgtcgaacctgcactgcatcggctcgcagggcatgggaccgtgggtgttcgaccgctggctggcccgcatcgtgatgtcgaagttcaagcacccgaagatcccgtcgctctcgacctcggacctagagtcgaacatcccgaacgagctgttcgacgccgagggcgacatggtgcgcgccatcaagaagctggactacaaggaccatgacggtgactataaagatcacgatatagattacaaggatgacgatgacaagtgacttaagggtaccggtgataccagcatcgtcttgatgccctggcagcaccctgctaaggaggcaacaagatgcataccatctaccgcatcgagaagaaggagaactacgtggtgctggacaagggcttcctgcacgaccgcgagctgtcgtggcaggctaagggcctgctggccttcatgctgtcgatgccgaacgactgggtgttcaacatgaaggacctccagaaccgctcgaagaacggtcgcgacgccacctaccgcattatgaaggagctgatcgaggccggctacgtgacccgcgtggagaaccgcgacggcggcaagttcggcaaggtggagtacgtggtccacgaggtgaagcagtcgccgcacaccgagtcgccggacaccgtgccgccctgcaccgagaacccgtaccccggcaacccgtaccccggcaacccgtacccggagaacccgccgctgctgaacaacaacaacaccaactacaagaacaccaacaacgacgacgacaacaaggaccgcccgaagaccaactcgctgaacgcctttcgcttctacgaggagaacttccagccgaccctgtcgtcggtggacatcgagatcctgaactactggctggaccgcttcccggaggagatcgtgctgtgcgccatgcggaaggccctagagcagaacgtgcgctcgatcaagtacatcgaccgcatccttgccaactgggagatgcagaaggtgcagacccttgaggacgtggcccgcctcgaccgccagtacgagctggagaagcaggcccgccagaagcgcggcggcgtggtgaacggctcggtccaccagcaccgcggctcggacggtcgctcgacgaaggaggacgagcgcatctcgcactacgagccgggcaagtgggacgacgtggacatctcgctggacggcctgctgcaccatcaccaccatcactgaacgcgtatcgat

SEQ ID NO: 16 - RNA, 3554 nt, Artificial Sequence
  RNA expression cassette for targets RdRp1, RdRp2, N protein and E protein
gcaugcggaucccugcagaguacucucuuauuguaacagcuuuaagggccaauucugcugucaaauuacagaauaaugagcuuaguccuguugcacuacgacagaugucuugugcugccgguacuacacaaacugcuugcacugaugacaaugcguuagcuuacuacaacacaacaaagggagguagguuuguacuugcacuguuauccgauuuacaggauuugaaaugggcuaguacucagcuggaaaugcugguauuguugguguacugacauuagauaaucaagaucucaaugguaacugguaugauuucggugauuucauacaaaccacgccagguaguggaguuccuguuguagauucuuauuauucauuguuaaugccuauauuaaccuugaccagggcuuuaacugcagagucacauguugacacugacuuaacaaagccuuacacagcuggauaucuuuagauuucaucuaaacgaacaaacuaaaaugucugauaauggaccccaaaaucagcgaaaugcaccccgcauuacguuugguggacccucagauucaacuggcaguaaccagaauggagaacgcaguggggcgcgaucaaaacaacgucggccccaagguuuacccaauaauacugcgucuugguucaccgcucucacucaacauggcaaggaagaccuuaaauucccucgaggacaaggcguuccaauuaacaccaauagcaguccagaugaccaaauuggcuacuaccgaagagcuaccagacgaauucgugguggugacgguaaaaugaaagaucucaguccaagaugguauuucuacuaccuaggaacugggccagaagcuggacuucccuauggugcuaacaaagacggcaucauauggguugcaacugagggagccuugaauacaccaaaagaucacauuggcacccgcaauccugcuaacaaugcugcaaucgugcuacaacuuccucaaggaacaacauugccaaaaggcuucuacgcagaagggagcagaggcggcagucaagccucuucucguuccucaucacguagucgcaacaguucaagaaauucaacuccaggcagcaguaggggaacuucuccugcuagaauggcuggcaauggcggugaugcugcucuugcuuugcugcugcuugacagauugaaccagcuugagagcaaaaugucugguaaaggccaacaacaacaaggccaaacugucacuaagaaaucugcugcugaggcuucuaagaagccucggcaaaaacguacugccacuaaagcauacaauguaacacaagcuuucggcagacgugguccagaacaaacccaaggaaauuuuggggaccaggaacuaaucagacaaggaacugauuacaaacauuggccgcaaauugcacaauuugcccccagcgcuucagcguucuucggaaugucgcgcauuggcauggaagucacaccuucgggaacgugguugaccuacacaggugccaucaaauuggaugacaaagauccaaauuucaaagaucaagucauuuugcugaauaagcauaugauaucuacguacucauucguuucggaagagacagguacguuaauaguuaauagcguacuucuuuuucuugcuuucgugguauucuugcuaguuacacuagccauccuuacugcgcuucgauugugugcguacugcugcaauauuguuaacgugagucuuguaaaaccuucuuuuuacguuuacucucguguuaaaaaucugaauucuucuagaguuccugaucuucuggucuaauacguaaagcuuaggaaggaauguacauauggcgaccgagggcgcgcgcaacaucggccagucggccccggagggcaaggugcagauggacugcccgucgcgccacaacuucgacccggagugcgagaaggcguuuguggagcacauccaccuugagcuggccucgucguaccacgcauggucgaugugggccuucuacgcccgcgacugcaaggccgccgugggcaugacccgccugugcgagugggccucgcacgucucggcccagcgcgcccgccgcauggccgccuacgugcugacccgcggcggccacguggacuacaaggagaucccggccccgaagaagcagggcugggacaacuucgaggacgccuucucgcacugcguggcgaacaagaagcgcauccugaccucgcuccagucgcuguaccagugcugccagucgaaggacgcccacugcucgaacuucauccagaccgacaugauggacgaggugaucgcguggaacaaguuucugucggacugccugucgaaccugcacugcaucggcucgcagggcaugggaccguggguguucgaccgcuggcuggcccgcaucgugaugucgaaguucaagcacccgaagaucccgucgcucucgaccucggaccuagagucgaacaucccgaacgagcuguucgacgccgagggcgacauggugcgcgccaucaagaagcuggacuacaaggaccaugacggugacuauaaagaucacgauauagauuacaaggaugacgaugacaagugacuuaaggguaccggugauaccagcaucgucuugaugcccuggcagcacccugcuaaggaggcaacaagaugcauaccaucuaccgcaucgagaagaaggagaacuacguggugcuggacaagggcuuccugcacgaccgcgagcugucguggcaggcuaagggccugcuggccuucaugcugucgaugccgaacgacuggguguucaacaugaaggaccuccagaaccgcucgaagaacggucgcgacgccaccuaccgcauuaugaaggagcugaucgaggccggcuacgugacccgcguggagaaccgcgacggcggcaaguucggcaagguggaguacgugguccacgaggugaagcagucgccgcacaccgagucgccggacaccgugccgcccugcaccgagaacccguaccccggcaacccguaccccggcaacccguacccggagaacccgccgcugcugaacaacaacaacaccaacuacaagaacaccaacaacgacgacgacaacaaggaccgcccgaagaccaacucgcugaacgccuuucgcuucuacgaggagaacuuccagccgacccugucgucgguggacaucgagauccugaacuacuggcuggaccgcuucccggaggagaucgugcugugcgccaugcggaaggcccuagagcagaacgugcgcucgaucaaguacaucgaccgcauccuugccaacugggagaugcagaaggugcagacccuugaggacguggcccgccucgaccgccaguacgagcuggagaagcaggcccgccagaagcgcggcggcguggugaacggcucgguccaccagcaccgcggcucggacggucgcucgacgaaggaggacgagcgcaucucgcacuacgagccgggcaagugggacgacguggacaucucgcuggacggccugcugcaccaucaccaccaucacugaacgcguaucgau

SEQ ID NO: 17 - RNA, 4302 nt, Artificial Sequence
  RNA expression cassette for targets Spike protein, ORF1ab 5' region, RdRp1, RdRp2, N protein and E protein
gcaugcggaucucgacacuugaacagcccuauguguucaucaaacguucggaugcucgaacugcaccucauggucauguuaugguugagcugguagcagaacucgaaggcauucaguacggucguaguggugagacacuugguguccuugucccucaugugggcgaaauaccaguggcuuaccgcaagguucuucuucguaagaacgguaauaaaggagcugguggccauaguuacggcgccgaucuaaagucauuugacuuaggcgacgagcuuggcacugauccuuaugaagauuuucaagaaaacuggaacacuaaacauagcagugguguuacccgugaacucaugcgugagcuuaacggaggggcauacacucgcuaugucgauaacaacuucuguggcccugauggcuacaagcuuaaauugauugccaaccaauuuaauagugcuauuggcaaaauucaagacucacuuucuuccacagcaagugcacuuggaaaacuucaagauguggucaaccaaaaugcacaagcuuuaaacacgcuuguuaaacaacuuagcuccaauuuuggugcaauuucaaguguuuuaaaugauauccuuucacgucuugacaaaguugaggcugaagugcaaauugauagguugaucacaggcagacuucaaaguuugcagacauaugugacucaacaauuaauuagagcugcagaaaucagagcuucugcuaaucuugcugcuacuaaaauguagaucgaucccugcagaguacucucuuauuguaacagcuuuaagggccaauucugcugucaaauuacagaauaaugagcuuaguccuguugcacuacgacagaugucuugugcugccgguacuacacaaacugcuugcacugaugacaaugcguuagcuuacuacaacacaacaaagggagguagguuuguacuugcacuguuauccgauuuacaggauuugaaaugggcuaguacucagcuggaaaugcugguauuguugguguacugacauuagauaaucaagaucucaaugguaacugguaugauuucggugauuucauacaaaccacgccagguaguggaguuccuguuguagauucuuauuauucauuguuaaugccuauauuaaccuugaccagggcuuuaacugcagagucacauguugacacugacuuaacaaagccuuacacagcuggauaucuuuagauuucaucuaaacgaacaaacuaaaaugucugauaauggaccccaaaaucagcgaaaugcaccccgcauuacguuugguggacccucagauucaacuggcaguaaccagaauggagaacgcaguggggcgcgaucaaaacaacgucggccccaagguuuacccaauaauacugcgucuugguucaccgcucucacucaacauggcaaggaagaccuuaaauucccucgaggacaaggcguuccaauuaacaccaauagcaguccagaugaccaaauuggcuacuaccgaagagcuaccagacgaauucgugguggugacgguaaaaugaaagaucucaguccaagaugguauuucuacuaccuaggaacugggccagaagcuggacuucccuauggugcuaacaaagacggcaucauauggguugcaacugagggagccuugaauacaccaaaagaucacauuggcacccgcaauccugcuaacaaugcugcaaucgugcuacaacuuccucaaggaacaacauugccaaaaggcuucuacgcagaagggagcagaggcggcagucaagccucuucucguuccucaucacguagucgcaacaguucaagaaauucaacuccaggcagcaguaggggaacuucuccugcuagaauggcuggcaauggcggugaugcugcucuugcuuugcugcugcuugacagauugaaccagcuugagagcaaaaugucugguaaaggccaacaacaacaaggccaaacugucacuaagaaaucugcugcugaggcuucuaagaagccucggcaaaaacguacugccacuaaagcauacaauguaacacaagcuuucggcagacgugguccagaacaaacccaaggaaauuuuggggaccaggaacuaaucagacaaggaacugauuacaaacauuggccgcaaauugcacaauuugcccccagcgcuucagcguucuucggaaugucgcgcauuggcauggaagucacaccuucgggaacgugguugaccuacacaggugccaucaaauuggaugacaaagauccaaauuucaaagaucaagucauuuugcugaauaagcauaugauaucuacguacucauucguuucggaagagacagguacguuaauaguuaauagcguacuucuuuuucuugcuuucgugguauucuugcuaguuacacuagccauccuuacugcgcuucgauugugugcguacugcugcaauauuguuaacgugagucuuguaaaaccuucuuuuuacguuuacucucguguuaaaaaucugaauucuucuagaguuccugaucuucuggucuaauacguaaagcuuaggaaggaauguacauauggcgaccgagggcgcgcgcaacaucggccagucggccccggagggcaaggugcagauggacugcccgucgcgccacaacuucgacccggagugcgagaaggcguuuguggagcacauccaccuugagcuggccucgucguaccacgcauggucgaugugggccuucuacgcccgcgacugcaaggccgccgugggcaugacccgccugugcgagugggccucgcacgucucggcccagcgcgcccgccgcauggccgccuacgugcugacccgcggcggccacguggacuacaaggagaucccggccccgaagaagcagggcugggacaacuucgaggacgccuucucgcacugcguggcgaacaagaagcgcauccugaccucgcuccagucgcuguaccagugcugccagucgaaggacgcccacugcucgaacuucauccagaccgacaugauggacgaggugaucgcguggaacaaguuucugucggacugccugucgaaccugcacugcaucggcucgcagggcaugggaccguggguguucgaccgcuggcuggcccgcaucgugaugucgaaguucaagcacccgaagaucccgucgcucucgaccucggaccuagagucgaacaucccgaacgagcuguucgacgccgagggcgacauggugcgcgccaucaagaagcuggacuacaaggaccaugacggugacuauaaagaucacgauauagauuacaaggaugacgaugacaagugacuuaaggguaccggugauaccagcaucgucuugaugcccuggcagcacccugcuaaggaggcaacaagaugcauaccaucuaccgcaucgagaagaaggagaacuacguggugcuggacaagggcuuccugcacgaccgcgagcugucguggcaggcuaagggccugcuggccuucaugcugucgaugccgaacgacuggguguucaacaugaaggaccuccagaaccgcucgaagaacggucgcgacgccaccuaccgcauuaugaaggagcugaucgaggccggcuacgugacccgcguggagaaccgcgacggcggcaaguucggcaagguggaguacgugguccacgaggugaagcagucgccgcacaccgagucgccggacaccgugccgcccugcaccgagaacccguaccccggcaacccguaccccggcaacccguacccggagaacccgccgcugcugaacaacaacaacaccaacuacaagaacaccaacaacgacgacgacaacaaggaccgcccgaagaccaacucgcugaacgccuuucgcuucuacgaggagaacuuccagccgacccugucgucgguggacaucgagauccugaacuacuggcuggaccgcuucccggaggagaucgugcugugcgccaugcggaaggcccuagagcagaacgugcgcucgaucaaguacaucgaccgcauccuugccaacugggagaugcagaaggugcagacccuugaggacguggcccgccucgaccgccaguacgagcuggagaagcaggcccgccagaagcgcggcggcguggugaacggcucgguccaccagcaccgcggcucggacggucgcucgacgaaggaggacgagcgcaucucgcacuacgagccgggcaagugggacgacguggacaucucgcuggacggccugcugcaccaucaccaccaucacugaacgcguaucgau

SEQ ID NO: 18 - DNA, 3100 bp, SARS-CoV-2
attaaaggtttataccttcccaggtaacaaaccaaccaactttcgatctcttgtagatctgttctctaaacgaactttaaaatctgtgtggctgtcactcggctgcatgcttagtgcactcacgcagtataattaataactaattactgtcgttgacaggacacgagtaactcgtctatcttctgcaggctgcttacggtttcgtccgtgttgcagccgatcatcagcacatctaggtttcgtccgggtgtgaccgaaaggtaagatggagagccttgtccctggtttcaacgagaaaacacacgtccaactcagtttgcctgttttacaggttcgcgacgtgctcgtacgtggctttggagactccgtggaggaggtcttatcagaggcacgtcaacatcttaaagatggcacttgtggcttagtagaagttgaaaaaggcgttttgcctcaacttgaacagccctatgtgttcatcaaacgttcggatgctcgaactgcacctcatggtcatgttatggttgagctggtagcagaactcgaaggcattcagtacggtcgtagtggtgagacacttggtgtccttgtccctcatgtgggcgaaataccagtggcttaccgcaaggttcttcttcgtaagaacggtaataaaggagctggtggccatagttacggcgccgatctaaagtcatttgacttaggcgacgagcttggcactgatccttatgaagattttcaagaaaactggaacactaaacatagcagtggtgttacccgtgaactcatgcgtgagcttaacggaggggcatacactcgctatgtcgataacaacttctgtggccctgatggctaccctcttgagtgcattaaagaccttctagcacgtgctggtaaagcttcatgcactttgtccgaacaactggactttattgacactaagaggggtgtatactgctgccgtgaacatgagcatgaaattgcttggtacacggaacgttctgaaaagagctatgaattgcagacaccttttgaaattaaattggcaaagaaatttgacaccttcaatggggaatgtccaaattttgtatttcccttaaattccataatcaagactattcaaccaagggttgaaaagaaaaagcttgatggctttatgggtagaattcgatctgtctatccagttgcgtcaccaaatgaatgcaaccaaatgtgcctttcaactctcatgaagtgtgatcattgtggtgaaacttcatggcagacgggcgattttgttaaagccacttgcgaattttgtggcactgagaatttgactaaagaaggtgccactacttgtggttacttaccccaaaatgctgttgttaaaatttattgtccagcatgtcacaattcagaagtaggacctgagcatagtcttgccgaataccataatgaatctggcttgaaaaccattcttcgtaagggtggtcgcactattgcctttggaggctgtgtgttctcttatgttggttgccataacaagtgtgcctattgggttccacgtgctagcgctaacataggttgtaaccatacaggtgttgttggagaaggttccgaaggtcttaatgacaaccttcttgaaatactccaaaaagagaaagtcaacatcaatattgttggtgactttaaacttaatgaagagatcgccattattttggcatctttttctgcttccacaagtgcttttgtggaaactgtgaaaggtttggattataaagcattcaaacaaattgttgaatcctgtggtaattttaaagttacaaaaggaaaagctaaaaaaggtgcctggaatattggtgaacagaaatcaatactgagtcctctttatgcatttgcatcagaggctgctcgtgttgtacgatcaattttctcccgcactcttgaaactgctcaaaattctgtgcgtgttttacagaaggccgctataacaatactagatggaatttcacagtattcactgagactcattgatgctatgatgttcacatctgatttggctactaacaatctagttgtaatggcctacattacaggtggtgttgttcagttgacttcgcagtggctaactaacatctttggcactgtttatgaaaaactcaaacccgtccttgattggcttgaagagaagtttaaggaaggtgtagagtttcttagagacggttgggaaattgttaaatttatctcaacctgtgcttgtgaaattgtcggtggacaaattgtcacctgtgcaaaggaaattaaggagagtgttcagacattctttaagcttgtaaataaatttttggctttgtgtgctgactctatcattattggtggagctaaacttaaagccttgaatttaggtgaaacatttgtcacgcactcaaagggattgtacagaaagtgtgttaaatccagagaagaaactggcctactcatgcctctaaaagccccaaaagaaattatcttcttagagggagaaacacttcccacagaagtgttaacagaggaagttgtcttgaaaactggtgatttacaaccattagaacaacctactagtgaagctgttgaagctccattggttggtacaccagtttgtattaacgggcttatgttgctcgaaatcaaagacacagaaaagtactgtgcccttgcacctaatatgatggtaacaaacaataccttcacactcaaaggcggtgcaccaacaaaggttacttttggtgatgacactgtgatagaagtgcaaggttacaagagtgtgaatatcacttttgaacttgatgaaaggattgataaagtacttaatgagaagtgctctgcctatacagttgaactcggtacagaagtaaatgagttcgcctgtgttgtggcagatgctgtcataaaaactttgcaaccagtatctgaattacttacaccactgggcattgatttagatgagtggagtatggctacatactacttatttgatgagtctggtgagtttaaattggcttcacatatgtattgttctttctaccctccagatgaggatgaagaagaaggtgattgtgaagaagaagagtttgagccatcaact

SEQ ID NO: 19 - DNA, 3070 bp, SARS-CoV-2
cttcacactcaaaggcggtgcaccaacaaaggttacttttggtgatgacactgtgatagaagtgcaaggttacaagagtgtgaatatcacttttgaacttgatgaaaggattgataaagtacttaatgagaagtgctctgcctatacagttgaactcggtacagaagtaaatgagttcgcctgtgttgtggcagatgctgtcataaaaactttgcaaccagtatctgaattacttacaccactgggcattgatttagatgagtggagtatggctacatactacttatttgatgagtctggtgagtttaaattggcttcacatatgtattgttctttctaccctccagatgaggatgaagaagaaggtgattgtgaagaagaagagtttgagccatcaactcaatatgagtatggtactgaagatgattaccaaggtaaacctttggaatttggtgccacttctgctgctcttcaacctgaagaagagcaagaagaagattggttagatgatgatagtcaacaaactgttggtcaacaagacggcagtgaggacaatcagacaactactattcaaacaattgttgaggttcaacctcaattagagatggaacttacaccagttgttcagactattgaagtgaatagttttagtggttatttaaaacttactgacaatgtatacattaaaaatgcagacattgtggaagaagctaaaaaggtaaaaccaacagtggttgttaatgcagccaatgtttaccttaaacatggaggaggtgttgcaggagccttaaataaggctactaacaatgccatgcaagttgaatctgatgattacatagctactaatggaccacttaaagtgggtggtagttgtgttttaagcggacacaatcttgctaaacactgtcttcatgttgtcggcccaaatgttaacaaaggtgaagacattcaacttcttaagagtgcttatgaaaattttaatcagcacgaagttctacttgcaccattattatcagctggtatttttggtgctgaccctatacattctttaagagtttgtgtagatactgttcgcacaaatgtctacttagctgtctttgataaaaatctctatgacaaacttgtttcaagctttttggaaatgaagagtgaaaagcaagttgaacaaaagatcgctgagattcctaaagaggaagttaagccatttataactgaaagtaaaccttcagttgaacagagaaaacaagatgataagaaaatcaaagcttgtgttgaagaagttacaacaactctggaagaaactaagttcctcacagaaaacttgttactttatattgacattaatggcaatcttcatccagattctgccactcttgttagtgacattgacatcactttcttaaagaaagatgctccatatatagtgggtgatgttgttcaagagggtgttttaactgctgtggttatacctactaaaaaggctggtggcactactgaaatgctagcgaaagctttgagaaaagtgccaacagacaattatataaccacttacccgggtcagggtttaaatggttacactgtagaggaggcaaagacagtgcttaaaaagtgtaaaagtgccttttacattctaccatctattatctctaatgagaagcaagaaattcttggaactgtttcttggaatttgcgagaaatgcttgcacatgcagaagaaacacgcaaattaatgcctgtctgtgtggaaactaaagccatagtttcaactatacagcgtaaatataagggtattaaaatacaagagggtgtggttgattatggtgctagattttacttttacaccagtaaaacaactgtagcgtcacttatcaacacacttaacgatctaaatgaaactcttgttacaatgccacttggctatgtaacacatggcttaaatttggaagaagctgctcggtatatgagatctctcaaagtgccagctacagtttctgtttcttcacctgatgctgttacagcgtataatggttatcttacttcttcttctaaaacacctgaagaacattttattgaaaccatctcacttgctggttcctataaagattggtcctattctggacaatctacacaactaggtatagaatttcttaagagaggtgataaaagtgtatattacactagtaatcctaccacattccacctagatggtgaagttatcacctttgacaatcttaagacacttctttctttgagagaagtgaggactattaaggtgtttacaacagtagacaacattaacctccacacgcaagttgtggacatgtcaatgacatatggacaacagtttggtccaacttatttggatggagctgatgttactaaaataaaacctcataattcacatgaaggtaaaacattttatgttttacctaatgatgacactctacgtgttgaggcttttgagtactaccacacaactgatcctagttttctgggtaggtacatgtcagcattaaatcacactaaaaagtggaaatacccacaagttaatggtttaacttctattaaatgggcagataacaactgttatcttgccactgcattgttaacactccaacaaatagagttgaagtttaatccacctgctctacaagatgcttattacagagcaagggctggtgaagctgctaacttttgtgcacttatcttagcctactgtaataagacagtaggtgagttaggtgatgttagagaaacaatgagttacttgtttcaacatgccaatttagattcttgcaaaagagtcttgaacgtggtgtgtaaaacttgtggacaacagcagacaacccttaagggtgtagaagctgttatgtacatgggcacactttcttatgaacaatttaagaaaggtgttcagataccttgtacgtgtggtaaacaagctacaaaatatctagtacaacaggagtcaccttttgttatgatgtcagcaccacctgctcagtatgaacttaagcatggtacatttacttgtgctagtgagtacactggtaattaccagtgtggtcac

SEQ ID NO: 20 - DNA, 3156 bp, SARS-CoV-2
acttatcttagcctactgtaataagacagtaggtgagttaggtgatgttagagaaacaatgagttacttgtttcaacatgccaatttagattcttgcaaaagagtcttgaacgtggtgtgtaaaacttgtggacaacagcagacaacccttaagggtgtagaagctgttatgtacatgggcacactttcttatgaacaatttaagaaaggtgttcagataccttgtacgtgtggtaaacaagctacaaaatatctagtacaacaggagtcaccttttgttatgatgtcagcaccacctgctcagtatgaacttaagcatggtacatttacttgtgctagtgagtacactggtaattaccagtgtggtcactataaacatataacttctaaagaaactttgtattgcatagacggtgctttacttacaaagtcctcagaatacaaaggtcctattacggatgttttctacaaagaaaacagttacacaacaaccataaaaccagttacttataaattggatggtgttgtttgtacagaaattgaccctaagttggacaattattataagaaagacaattcttatttcacagagcaaccaattgatcttgtaccaaaccaaccatatccaaacgcaagcttcgataattttaagtttgtatgtgataatatcaaatttgctgatgatttaaaccagttaactggttataagaaacctgcttcaagagagcttaaagttacatttttccctgacttaaatggtgatgtggtggctattgattataaacactacacaccctcttttaagaaaggagctaaattgttacataaacctattgtttggcatgttaacaatgcaactaataaagccacgtataaaccaaatacctggtgtatacgttgtctttggagcacaaaaccagttgaaacatcaaattcgtttgatgtactgaagtcagaggacgcgcagggaatggataatcttgcctgcgaagatctaaaaccagtctctgaagaagtagtggaaaatcctaccatacagaaagacgttcttgagtgtaatgtgaaaactaccgaagttgtaggagacattatacttaaaccagcaaataatagtttaaaaattacagaagaggttggccacacagatctaatggctgcttatgtagacaattctagtcttactattaagaaacctaatgaattatctagagtattaggtttgaaaacccttgctactcatggtttagctgctgttaatagtgtcccttgggatactatagctaattatgctaagccttttcttaacaaagttgttagtacaactactaacatagttacacggtgtttaaaccgtgtttgtactaattatatgccttatttctttactttattgctacaattgtgtacttttactagaagtacaaattctagaattaaagcatctatgccgactactatagcaaagaatactgttaagagtgtcggtaaattttgtctagaggcttcatttaattatttgaagtcacctaatttttctaaactgataaatattataatttggtttttactattaagtgtttgcctaggttctttaatctactcaaccgctgctttaggtgttttaatgtctaatttaggcatgccttcttactgtactggttacagagaaggctatttgaactctactaatgtcactattgcaacctactgtactggttctataccttgtagtgtttgtcttagtggtttagattctttagacacctatccttctttagaaactatacaaattaccatttcatcttttaaatgggatttaactgcttttggcttagttgcagagtggtttttggcatatattcttttcactaggtttttctatgtacttggattggctgcaatcatgcaattgtttttcagctattttgcagtacattttattagtaattcttggcttatgtggttaataattaatcttgtacaaatggccccgatttcagctatggttagaatgtacatcttctttgcatcattttattatgtatggaaaagttatgtgcatgttgtagacggttgtaattcatcaacttgtatgatgtgttacaaacgtaatagagcaacaagagtcgaatgtacaactattgttaatggtgttagaaggtccttttatgtctatgctaatggaggtaaaggcttttgcaaactacacaattggaattgtgttaattgtgatacattctgtgctggtagtacatttattagtgatgaagttgcgagagacttgtcactacagtttaaaagaccaataaatcctactgaccagtcttcttacatcgttgatagtgttacagtgaagaatggttccatccatctttactttgataaagctggtcaaaagacttatgaaagacattctctctctcattttgttaacttagacaacctgagagctaataacactaaaggttcattgcctattaatgttatagtttttgatggtaaatcaaaatgtgaagaatcatctgcaaaatcagcgtctgtttactacagtcagcttatgtgtcaacctatactgttactagatcaggcattagtgtctgatgttggtgatagtgcggaagttgcagttaaaatgtttgatgcttacgttaatacgttttcatcaacttttaacgtaccaatggaaaaactcaaaacactagttgcaactgcagaagctgaacttgcaaagaatgtgtccttagacaatgtcttatctacttttatttcagcagctcggcaagggtttgttgattcagatgtagaaactaaagatgttgttgaatgtcttaaattgtcacatcaatctgacatagaagttactggcgatagttgtaataactatatgctcacctataacaaagttgaaaacatgacaccccgtgaccttggtgcttgtattgactgtagtgcgcgtcatattaatgcgcaggtagcaaaaagtcacaacattgctttgatatggaacgttaaagatttcatgtcattgtctgaacaactacgaaaacaaatacgtagtgctgctaaaaagaataacttaccttttaagttgacatgtgcaactactagacaagttgttaatgttgtaacaacaaagatagcacttaagggtggtaa

SEQ ID NO: 21 - DNA, 3105 bp, SARS-CoV-2
agttgcaactgcagaagctgaacttgcaaagaatgtgtccttagacaatgtcttatctacttttatttcagcagctcggcaagggtttgttgattcagatgtagaaactaaagatgttgttgaatgtcttaaattgtcacatcaatctgacatagaagttactggcgatagttgtaataactatatgctcacctataacaaagttgaaaacatgacaccccgtgaccttggtgcttgtattgactgtagtgcgcgtcatattaatgcgcaggtagcaaaaagtcacaacattgctttgatatggaacgttaaagatttcatgtcattgtctgaacaactacgaaaacaaatacgtagtgctgctaaaaagaataacttaccttttaagttgacatgtgcaactactagacaagttgttaatgttgtaacaacaaagatagcacttaagggtggtaaaattgttaataattggttgaagcagttaattaaagttacacttgtgttcctttttgttgctgctattttctatttaataacacctgttcatgtcatgtctaaacatactgacttttcaagtgaaatcataggatacaaggctattgatggtggtgtcactcgtgacatagcatctacagatacttgttttgctaacaaacatgctgattttgacacatggtttagccagcgtggtggtagttatactaatgacaaagcttgcccattgattgctgcagtcataacaagagaagtgggttttgtcgtgcctggtttgcctggcacgatattacgcacaactaatggtgactttttgcatttcttacctagagtttttagtgcagttggtaacatctgttacacaccatcaaaacttatagagtacactgactttgcaacatcagcttgtgttttggctgctgaatgtacaatttttaaagatgcttctggtaagccagtaccatattgttatgataccaatgtactagaaggttctgttgcttatgaaagtttacgccctgacacacgttatgtgctcatggatggctctattattcaatttcctaacacctaccttgaaggttctgttagagtggtaacaacttttgattctgagtactgtaggcacggcacttgtgaaagatcagaagctggtgtttgtgtatctactagtggtagatgggtacttaacaatgattattacagatctttaccaggagttttctgtggtgtagatgctgtaaatttacttactaatatgtttacaccactaattcaacctattggtgctttggacatatcagcatctatagtagctggtggtattgtagctatcgtagtaacatgccttgcctactattttatgaggtttagaagagcttttggtgaatacagtcatgtagttgcctttaatactttactattccttatgtcattcactgtactctgtttaacaccagtttactcattcttacctggtgtttattctgttatttacttgtacttgacattttatcttactaatgatgtttcttttttagcacatattcagtggatggttatgttcacacctttagtacctttctggataacaattgcttatatcatttgtatttccacaaagcatttctattggttctttagtaattacctaaagagacgtgtagtctttaatggtgtttcctttagtacttttgaagaagctgcgctgtgcacctttttgttaaataaagaaatgtatctaaagttgcgtagtgatgtgctattacctcttacgcaatataatagatacttagctctttataataagtacaagtattttagtggagcaatggatacaactagctacagagaagctgcttgttgtcatctcgcaaaggctctcaatgacttcagtaactcaggttctgatgttctttaccaaccaccacaaacctctatcacctcagctgttttgcagagtggttttagaaaaatggcattcccatctggtaaagttgagggttgtatggtacaagtaacttgtggtacaactacacttaacggtctttggcttgatgacgtagtttactgtccaagacatgtgatctgcacctctgaagacatgcttaaccctaattatgaagatttactcattcgtaagtctaatcataatttcttggtacaggctggtaatgttcaactcagggttattggacattctatgcaaaattgtgtacttaagcttaaggttgatacagccaatcctaagacacctaagtataagtttgttcgcattcaaccaggacagactttttcagtgttagcttgttacaatggttcaccatctggtgtttaccaatgtgctatgaggcccaatttcactattaagggttcattccttaatggttcatgtggtagtgttggttttaacatagattatgactgtgtctctttttgttacatgcaccatatggaattaccaactggagttcatgctggcacagacttagaaggtaacttttatggaccttttgttgacaggcaaacagcacaagcagctggtacggacacaactattacagttaatgttttagcttggttgtacgctgctgttataaatggagacaggtggtttctcaatcgatttaccacaactcttaatgactttaaccttgtggctatgaagtacaattatgaacctctaacacaagaccatgttgacatactaggacctctttctgctcaaactggaattgccgttttagatatgtgtgcttcattaaaagaattactgcaaaatggtatgaatggacgtaccatattgggtagtgctttattagaagatgaatttacaccttttgatgttgttagacaatgctcaggtgttactttccaaagtgcagtgaaaagaacaatcaagggtacacaccactggttgttactcacaattttgacttcacttttagttttagtccagagtactcaatggtctttgttcttttttttgtatgaaaatgcctttttaccttttgctatgggtattattgctatgtctgcttttgcaatgatgtttgtcaaacataagcatgcatttctctgtttgtttttgttaccttctcttgccactgt

SEQ ID NO: 22 - DNA, 3101 bp, SARS-CoV-2
actaggacctctttctgctcaaactggaattgccgttttagatatgtgtgcttcattaaaagaattactgcaaaatggtatgaatggacgtaccatattgggtagtgctttattagaagatgaatttacaccttttgatgttgttagacaatgctcaggtgttactttccaaagtgcagtgaaaagaacaatcaagggtacacaccactggttgttactcacaattttgacttcacttttagttttagtccagagtactcaatggtctttgttcttttttttgtatgaaaatgcctttttaccttttgctatgggtattattgctatgtctgcttttgcaatgatgtttgtcaaacataagcatgcatttctctgtttgtttttgttaccttctcttgccactgtagcttattttaatatggtctatatgcctgctagttgggtgatgcgtattatgacatggttggatatggttgatactagtttgtctggttttaagctaaaagactgtgttatgtatgcatcagctgtagtgttactaatccttatgacagcaagaactgtgtatgatgatggtgctaggagagtgtggacacttatgaatgtcttgacactcgtttataaagtttattatggtaatgctttagatcaagccatttccatgtgggctcttataatctctgttacttctaactactcaggtgtagttacaactgtcatgtttttggccagaggtattgtttttatgtgtgttgagtattgccctattttcttcataactggtaatacacttcagtgtataatgctagtttattgtttcttaggctatttttgtacttgttactttggcctcttttgtttactcaaccgctactttagactgactcttggtgtttatgattacttagtttctacacaggagtttagatatatgaattcacagggactactcccacccaagaatagcatagatgccttcaaactcaacattaaattgttgggtgttggtggcaaaccttgtatcaaagtagccactgtacagtctaaaatgtcagatgtaaagtgcacatcagtagtcttactctcagttttgcaacaactcagagtagaatcatcatctaaattgtgggctcaatgtgtccagttacacaatgacattctcttagctaaagatactactgaagcctttgaaaaaatggtttcactactttctgttttgctttccatgcagggtgctgtagacataaacaagctttgtgaagaaatgctggacaacagggcaaccttacaagctatagcctcagagtttagttcccttccatcatatgcagcttttgctactgctcaagaagcttatgagcaggctgttgctaatggtgattctgaagttgttcttaaaaagttgaagaagtctttgaatgtggctaaatctgaatttgaccgtgatgcagccatgcaacgtaagttggaaaagatggctgatcaagctatgacccaaatgtataaacaggctagatctgaggacaagagggcaaaagttactagtgctatgcagacaatgcttttcactatgcttagaaagttggataatgatgcactcaacaacattatcaacaatgcaagagatggttgtgttcccttgaacataatacctcttacaacagcagccaaactaatggttgtcataccagactataacacatataaaaatacgtgtgatggtacaacatttacttatgcatcagcattgtgggaaatccaacaggttgtagatgcagatagtaaaattgttcaacttagtgaaattagtatggacaattcacctaatttagcatggcctcttattgtaacagctttaagggccaattctgctgtcaaattacagaataatgagcttagtcctgttgcactacgacagatgtcttgtgctgccggtactacacaaactgcttgcactgatgacaatgcgttagcttactacaacacaacaaagggaggtaggtttgtacttgcactgttatccgatttacaggatttgaaatgggctagattccctaagagtgatggaactggtactatctatacagaactggaaccaccttgtaggtttgttacagacacacctaaaggtcctaaagtgaagtatttatactttattaaaggattaaacaacctaaatagaggtatggtacttggtagtttagctgccacagtacgtctacaagctggtaatgcaacagaagtgcctgccaattcaactgtattatctttctgtgcttttgctgtagatgctgctaaagcttacaaagattatctagctagtgggggacaaccaatcactaattgtgttaagatgttgtgtacacacactggtactggtcaggcaataacagttacaccggaagccaatatggatcaagaatcctttggtggtgcatcgtgttgtctgtactgccgttgccacatagatcatccaaatcctaaaggattttgtgacttaaaaggtaagtatgtacaaatacctacaacttgtgctaatgaccctgtgggttttacacttaaaaacacagtctgtaccgtctgcggtatgtggaaaggttatggctgtagttgtgatcaactccgcgaacccatgcttcagtcagctgatgcacaatcgtttttaaacgggtttgcggtgtaagtgcagcccgtcttacaccgtgcggcacaggcactagtactgatgtcgtatacagggcttttgacatctacaatgataaagtagctggttttgctaaattcctaaaaactaattgttgtcgcttccaagaaaaggacgaagatgacaatttaattgattcttactttgtagttaagagacacactttctctaactaccaacatgaagaaacaatttataatttacttaaggattgtccagctgttgctaaacatgacttctttaagtttagaatagacggtgacatggtaccacatatatcacgtcaacgtcttactaaatacacaatggcagacctcgtctatgctttaaggcattttgatgaaggtaattgtgacacattaaaagaaatacttgtcacatacaattgttgtgatga

SEQ ID NO: 23 - DNA, 2940 bp, SARS-CoV-2
gcgcggatccccgtgcggcacaggcactagtactgatgtcgtatacagggcttttgacatctacaatgataaagtagctggttttgctaaattcctaaaaactaattgttgtcgcttccaagaaaaggacgaagatgacaatttaattgattcttactttgtagttaagagacacactttctctaactaccaacatgaagaaacaatttataatttacttaaggattgtccagctgttgctaaacatgacttctttaagtttagaatagacggtgacatggtaccacatatatcacgtcaacgtcttactaaatacacaatggcagacctcgtctatgctttaaggcattttgatgaaggtaattgtgacacattaaaagaaatacttgtcacatacaattgttgtgatgatgattatttcaataaaaaggactggtatgattttgtagaaaacccagatatattacgcgtatacgccaacttaggtgaacgtgtacgccaagctttgttaaaaacagtacaattctgtgatgccatgcgaaatgctggtattgttggtgtactgacattagataatcaagatctcaatggtaactggtatgatttcggtgatttcatacaaaccacgccaggtagtggagttcctgttgtagattcttattattcattgttaatgcctatattaaccttgaccagggctttaactgcagagtcacatgttgacactgacttaacaaagccttacattaagtgggatttgttaaaatatgacttcacggaagagaggttaaaactctttgaccgttattttaaatattgggatcagacataccacccaaattgtgttaactgtttggatgacagatgcattctgcattgtgcaaactttaatgttttattctctacagtgttcccacctacaagttttggaccactagtgagaaaaatatttgttgatggtgttccatttgtagtttcaactggataccacttcagagagctaggtgttgtacataatcaggatgtaaacttacatagctctagacttagttttaaggaattacttgtgtatgctgctgaccctgctatgcacgctgcttctggtaatctattactagataaacgcactacgtgcttttcagtagctgcacttactaacaatgttgcttttcaaactgtcaaacccggtaattttaacaaagacttctatgactttgctgtgtctaagggtttctttaaggaaggaagttctgttgaattaaaacacttcttctttgctcaggatggtaatgctgctatcagcgattatgactactatcgttataatctaccaacaatgtgtgatatcagacaactactatttgtagttgaagttgttgataagtactttgattgttacgatggtggctgtattaatgctaaccaagtcatcgtcaacaacctagacaaatcagctggttttccatttaataaatggggtaaggctagactttattatgattcaatgagttatgaggatcaagatgcacttttcgcatatacaaaacgtaatgtcatccctactataactcaaatgaatcttaagtatgccattagtgcaaagaatagagctcgcaccgtagctggtgtctctatctgtagtactatgaccaatagacagtttcatcaaaaattattgaaatcaatagccgccactagaggagctactgtagtaattggaacaagcaaattctatggtggttggcacaacatgttaaaaactgtttatagtgatgtagaaaaccctcaccttatgggttgggattatcctaaatgtgatagagccatgcctaacatgcttagaattatggcctcacttgttcttgctcgcaaacatacaacgtgttgtagcttgtcacaccgtttctatagattagctaatgagtgtgctcaagtattgagtgaaatggtcatgtgtggcggttcactatatgttaaaccaggtggaacctcatcaggagatgccacaactgcttatgctaatagtgtttttaacatttgtcaagctgtcacggccaatgttaatgcacttttatctactgatggtaacaaaattgccgataagtatgtccgcaatttacaacacagactttatgagtgtctctatagaaatagagatgttgacacagactttgtgaatgagttttacgcatatttgcgtaaacatttctcaatgatgatactctctgacgatgctgttgtgtgtttcaatagcacttatgcatctcaaggtctagtggctagcataaagaactttaagtcagttctttattatcaaaacaatgtttttatgtctgaagcaaaatgttggactgagactgaccttactaaaggacctcatgaattttgctctcaacatacaatgctagttaaacagggtgatgattatgtgtaccttccttacccagatccatcaagaatcctaggggccggctgttttgtagatgatatcgtaaaaacagatggtacacttatgattgaacggttcgtgtctttagctatagatgcttacccacttactaaacatcctaatcaggagtatgctgatgtctttcatttgtacttacaatacataagaaagctacatgatgagttaacaggacacatgttagacatgtattctgttatgcttactaatgataacacttcaaggtattgggaacctgagttttatgaggctatgtacacaccgcatacagtcttacaggctgttggggcttgtgttctttgcaattcacagacttcattaagatgtggtgcttgcatacgtagaccattcttatgttgtaaatgctgttacgaccatgtcatatcaacatcacataaattagtcttgtctgttaatccgtatgtttgcaatgctccaggttgtgatgtcacagatgtgactctcgcgaggcc

SEQ ID NO: 24 - DNA, 3110 bp, SARS-CoV-2
tatgaggctatgtacacaccgcatacagtcttacaggctgttggggcttgtgttctttgcaattcacagacttcattaagatgtggtgcttgcatacgtagaccattcttatgttgtaaatgctgttacgaccatgtcatatcaacatcacataaattagtcttgtctgttaatccgtatgtttgcaatgctccaggttgtgatgtcacagatgtgactcaactttacttaggaggtatgagctattattgtaaatcacataaaccacccattagttttccattgtgtgctaatggacaagtttttggtttatataaaaatacatgtgttggtagcgataatgttactgactttaatgcaattgcaacatgtgactggacaaatgctggtgattacattttagctaacacctgtactgaaagactcaagctttttgcagcagaaacgctcaaagctactgaggagacatttaaactgtcttatggtattgctactgtacgtgaagtgctgtctgacagagaattacatctttcatgggaagttggtaaacctagaccaccacttaaccgaaattatgtctttactggttatcgtgtaactaaaaacagtaaagtacaaataggagagtacacctttgaaaaaggtgactatggtgatgctgttgtttaccgaggtacaacaacttacaaattaaatgttggtgattattttgtgctgacatcacatacagtaatgccattaagtgcacctacactagtgccacaagagcactatgttagaattactggcttatacccaacactcaatatctcagatgagttttctagcaatgttgcaaattatcaaaaggttggtatgcaaaagtattctacactccagggaccacctggtactggtaagagtcattttgctattggcctagctctctactacccttctgctcgcatagtgtatacagcttgctctcatgccgctgttgatgcactatgtgagaaggcattaaaatatttgcctatagataaatgtagtagaattatacctgcacgtgctcgtgtagagtgttttgataaattcaaagtgaattcaacattagaacagtatgtcttttgtactgtaaatgcattgcctgagacgacagcagatatagttgtctttgatgaaatttcaatggccacaaattatgatttgagtgttgtcaatgccagattacgtgctaagcactatgtgtacattggcgaccctgctcaattacctgcaccacgcacattgctaactaagggcacactagaaccagaatatttcaattcagtgtgtagacttatgaaaactataggtccagacatgttcctcggaacttgtcggcgttgtcctgctgaaattgttgacactgtgagtgctttggtttatgataataagcttaaagcacataaagacaaatcagctcaatgctttaaaatgttttataagggtgttatcacgcatgatgtttcatctgcaattaacaggccacaaataggcgtggtaagagaattccttacacgtaaccctgcttggagaaaagctgtctttatttcaccttataattcacagaatgctgtagcctcaaagattttgggactaccaactcaaactgttgattcatcacagggctcagaatatgactatgtcatattcactcaaaccactgaaacagctcactcttgtaatgtaaacagatttaatgttgctattaccagagcaaaagtaggcatactttgcataatgtctgatagagacctttatgacaagttgcaatttacaagtcttgaaattccacgtaggaatgtggcaactttacaagctgaaaatgtaacaggactctttaaagattgtagtaaggtaatcactgggttacatcctacacaggcacctacacacctcagtgttgacactaaattcaaaactgaaggtttatgtgttgacatacctggcatacctaaggacatgacctatagaagactcatctctatgatgggttttaaaatgaattatcaagttaatggttaccctaacatgtttatcacccgcgaagaagctataagacatgtacgtgcatggattggcttcgatgtcgaggggtgtcatgctactagagaagctgttggtaccaatttacctttacagctaggtttttctacaggtgttaacctagttgctgtacctacaggttatgttgatacacctaataatacagatttttccagagttagtgctaaaccaccgcctggagatcaatttaaacacctcataccacttatgtacaaaggacttccttggaatgtagtgcgtataaagattgtacaaatgttaagtgacacacttaaaaatctctctgacagagtcgtatttgtcttatgggcacatggctttgagttgacatctatgaagtattttgtgaaaataggacctgagcgcacctgttgtctatgtgatagacgtgccacatgcttttccactgcttcagacacttatgcctgttggcatcattctattggatttgattacgtctataatccgtttatgattgatgttcaacaatggggttttacaggtaacctacaaagcaaccatgatctgtattgtcaagtccatggtaatgcacatgtagctagttgtgatgcaatcatgactaggtgtctagctgtccacgagtgctttgttaagcgtgttgactggactattgaatatcctataattggtgatgaactgaagattaatgcggcttgtagaaaggttcaacacatggttgttaaagctgcattattagcagacaaattcccagttcttcacgacattggtaaccctaaagctattaagtgtgtacctcaagctgatgtagaatggaagttctatgatgcacagccttgtagtgacaaagcttataaaatagaagaattattctattcttatgccacacattctgacaaattcacagatggtgtatgcctattttggaattgcaatgtcgatagatatcctgctaattccattgtttgtagatttgacactagagtgctatctaaccttaacttgcctggttgtgatggtggcagtttgtatgtcgcgaggcc

SEQ ID NO: 25 - DNA, 3167 bp, SARS-CoV-2
gcgcggatccaagcgtgttgactggactattgaatatcctataattggtgatgaactgaagattaatgcggcttgtagaaaggttcaacacatggttgttaaagctgcattattagcagacaaattcccagttcttcacgacattggtaaccctaaagctattaagtgtgtacctcaagctgatgtagaatggaagttctatgatgcacagccttgtagtgacaaagcttataaaatagaagaattattctattcttatgccacacattctgacaaattcacagatggtgtatgcctattttggaattgcaatgtcgatagatatcctgctaattccattgtttgtagatttgacactagagtgctatctaaccttaacttgcctggttgtgatggtggcagtttgtatgtaaataaacatgcattccacacaccagcttttgataaaagtgcttttgttaatttaaaacaattaccatttttctattactctgacagtccatgtgagtctcatggaaaacaagtagtgtcagatatagattatgtaccactaaagtctgctacgtgtataacacgttgcaatttaggtggtgctgtctgtagacatcatgctaatgagtacagattgtatctcgatgcttataacatgatgatctcagctggctttagcttgtgggtttacaaacaatttgatacttataacctctggaacacttttacaagacttcagagtttagaaaatgtggcttttaatgttgtaaataagggacactttgatggacaacagggtgaagtaccagtttctatcattaataacactgtttacacaaaagttgatggtgttgatgtagaattgtttgaaaataaaacaacattacctgttaatgtagcatttgagctttgggctaagcgcaacattaaaccagtaccagaggtgaaaatactcaataatttgggtgtggacattgctgctaatactgtgatctgggactacaaaagagatgctccagcacatatatctactattggtgtttgttctatgactgacatagccaagaaaccaactgaaacgatttgtgcaccactcactgtcttttttgatggtagagttgatggtcaagtagacttatttagaaatgcccgtaatggtgttcttattacagaaggtagtgttaaaggtttacaaccatctgtaggtcccaaacaagctagtcttaatggagtcacattaattggagaagccgtaaaaacacagttcaattattataagaaagttgatggtgttgtccaacaattacctgaaacttactttactcagagtagaaatttacaagaatttaaacccaggagtcaaatggaaattgatttcttagaattagctatggatgaattcattgaacggtataaattagaaggctatgccttcgaacatatcgtttatggagattttagtcatagtcagttaggtggtttacatctactgattggactagctaaacgttttaaggaatcaccttttgaattagaagattttattcctatggacagtacagttaaaaactatttcataacagatgcgcaaacaggttcatctaagtgtgtgtgttctgttattgatttattacttgatgattttgttgaaataataaaatcccaagatttatctgtagtttctaaggttgtcaaagtgactattgactatacagaaatttcatttatgctttggtgtaaagatggccatgtagaaacattttacccaaaattacaatctagtcaagcgtggcaaccgggtgttgctatgcctaatctttacaaaatgcaaagaatgctattagaaaagtgtgaccttcaaaattatggtgatagtgcaacattacctaaaggcataatgatgaatgtcgcaaaatatactcaactgtgtcaatatttaaacacattaacattagctgtaccctataatatgagagttatacattttggtgctggttctgataaaggagttgcaccaggtacagctgttttaagacagtggttgcctacgggtacgctgcttgtcgattcagatcttaatgactttgtctctgatgcagattcaactttgattggtgattgtgcaactgtacatacagctaataaatgggatctcattattagtgatatgtacgaccctaagactaaaaatgttacaaaagaaaatgactctaaagagggttttttcacttacatttgtgggtttatacaacaaaagctagctcttggaggttccgtggctataaagataacagaacattcttggaatgctgatctttataagctcatgggacacttcgcatggtggacagcctttgttactaatgtgaatgcgtcatcatctgaagcatttttaattggatgtaattatcttggcaaaccacgcgaacaaatagatggttatgtcatgcatgcaaattacatattttggaggaatacaaatccaattcagttgtcttcctattctttatttgacatgagtaaatttccccttaaattaaggggtactgctgttatgtctttaaaagaaggtcaaatcaatgatatgattttatctcttcttagtaaaggtagacttataattagagaaaacaacagagttgttatttctagtgatgttcttgttaacaactaaacgaacaatgtttgtttttcttgttttattgccactagtctctagtcagtgtgttaatcttacaaccagaactcaattaccccctgcatacactaattctttcacacgtggtgtttattaccctgacaaagttttcagatcctcagttttacattcaactcaggacttgttcttacctttcttttccaatgttacttggttccatgctatacatgtctctgggaccaatggtactaagaggtttgataaccctgtcctaccatttaatgatggtgtttattttgcttccactgagaagtctaacataataagaggctggatttttggtactactttagattcgaagacccagtccctacttattgttaataacgctactaatgttgttattaaagtctgtgaatttcaattttgtaatgatccatttttgggtgtttattaccacaaaaacaacaaaagttggatggaaagtgagttcagagtttattctagtacgtaggcc

SEQ ID NO: 26 - DNA, 3117 bp, SARS-CoV-2
tcagtgtgttaatcttacaaccagaactcaattaccccctgcatacactaattctttcacacgtggtgtttattaccctgacaaagttttcagatcctcagttttacattcaactcaggacttgttcttacctttcttttccaatgttacttggttccatgctatacatgtctctgggaccaatggtactaagaggtttgataaccctgtcctaccatttaatgatggtgtttattttgcttccactgagaagtctaacataataagaggctggatttttggtactactttagattcgaagacccagtccctacttattgttaataacgctactaatgttgttattaaagtctgtgaatttcaattttgtaatgatccatttttgggtgtttattaccacaaaaacaacaaaagttggatggaaagtgagttcagagtttattctagtgcgaataattgcacttttgaatatgtctctcagccttttcttatggaccttgaaggaaaacagggtaatttcaaaaatcttagggaatttgtgtttaagaatattgatggttattttaaaatatattctaagcacacgcctattaatttagtgcgtgatctccctcagggtttttcggctttagaaccattggtagatttgccaataggtattaacatcactaggtttcaaactttacttgctttacatagaagttatttgactcctggtgattcttcttcaggttggacagctggtgctgcagcttattatgtgggttatcttcaacctaggacttttctattaaaatataatgaaaatggaaccattacagatgctgtagactgtgcacttgaccctctctcagaaacaaagtgtacgttgaaatccttcactgtagaaaaaggaatctatcaaacttctaactttagagtccaaccaacagaatctattgttagatttcctaatattacaaacttgtgcccttttggtgaagtttttaacgccaccagatttgcatctgtttatgcttggaacaggaagagaatcagcaactgtgttgctgattattctgtcctatataattccgcatcattttccacttttaagtgttatggagtgtctcctactaaattaaatgatctctgctttactaatgtctatgcagattcatttgtaattagaggtgatgaagtcagacaaatcgctccagggcaaactggaaagattgctgattataattataaattaccagatgattttacaggctgcgttatagcttggaattctaacaatcttgattctaaggttggtggtaattataattacctgtatagattgtttaggaagtctaatctcaaaccttttgagagagatatttcaactgaaatctatcaggccggtagcacaccttgtaatggtgttgaaggttttaattgttactttcctttacaatcatatggtttccaacccactaatggtgttggttaccaaccatacagagtagtagtactttcttttgaacttctacatgcaccagcaactgtttgtggacctaaaaagtctactaatttggttaaaaacaaatgtgtcaatttcaacttcaatggtttaacaggcacaggtgttcttactgagtctaacaaaaagtttctgcctttccaacaatttggcagagacattgctgacactactgatgctgtccgtgatccacagacacttgagattcttgacattacaccatgttcttttggtggtgtcagtgttataacaccaggaacaaatacttctaaccaggttgctgttctttatcaggatgttaactgcacagaagtccctgttgctattcatgcagatcaacttactcctacttggcgtgtttattctacaggttctaatgtttttcaaacacgtgcaggctgtttaataggggctgaacatgtcaacaactcatatgagtgtgacatacccattggtgcaggtatatgcgctagttatcagactcagactaattctcctcggcgggcacgtagtgtagctagtcaatccatcattgcctacactatgtcacttggtgcagaaaattcagttgcttactctaataactctattgccatacccacaaattttactattagtgttaccacagaaattctaccagtgtctatgaccaagacatcagtagattgtacaatgtacatttgtggtgattcaactgaatgcagcaatcttttgttgcaatatggcagtttttgtacacaattaaaccgtgctttaactggaatagctgttgaacaagacaaaaacacccaagaagtttttgcacaagtcaaacaaatttacaaaacaccaccaattaaagattttggtggttttaatttttcacaaatattaccagatccatcaaaaccaagcaagaggtcatttattgaagatctacttttcaacaaagtgacacttgcagatgctggcttcatcaaacaatatggtgattgccttggtgatattgctgctagagacctcatttgtgcacaaaagtttaacggccttactgttttgccacctttgctcacagatgaaatgattgctcaatacacttctgcactgttagcgggtacaatcacttctggttggacctttggtgcaggtgctgcattacaaataccatttgctatgcaaatggcttataggtttaatggtattggagttacacagaatgttctctatgagaaccaaaaattgattgccaaccaatttaatagtgctattggcaaaattcaagactcactttcttccacagcaagtgcacttggaaaacttcaagatgtggtcaaccaaaatgcacaagctttaaacacgcttgttaaacaacttagctccaattttggtgcaatttcaagtgttttaaatgatatcctttcacgtcttgacaaagttgaggctgaagtgcaaattgataggttgatcacaggcagacttcaaagtttgcagacatatgtgactcaacaattaattagagctgcagaaatcagagcttctgctaatcttgctgctactaaaatgtcagagtgtgtacttggacaatcaaaaagagttgatttttgtggaaagggctatcatcttatgtcctt

SEQ ID NO: 27 - DNA, 2863 bp, SARS-CoV-2
gaatgttctctatgagaaccaaaaattgattgccaaccaatttaatagtgctattggcaaaattcaagactcactttcttccacagcaagtgcacttggaaaacttcaagatgtggtcaaccaaaatgcacaagctttaaacacgcttgttaaacaacttagctccaattttggtgcaatttcaagtgttttaaatgatatcctttcacgtcttgacaaagttgaggctgaagtgcaaattgataggttgatcacaggcagacttcaaagtttgcagacatatgtgactcaacaattaattagagctgcagaaatcagagcttctgctaatcttgctgctactaaaatgtcagagtgtgtacttggacaatcaaaaagagttgatttttgtggaaagggctatcatcttatgtccttccctcagtcagcacctcatggtgtagtcttcttgcatgtgacttatgtccctgcacaagaaaagaacttcacaactgctcctgccatttgtcatgatggaaaagcacactttcctcgtgaaggtgtctttgtttcaaatggcacacactggtttgtaacacaaaggaatttttatgaaccacaaatcattactacagacaacacatttgtgtctggtaactgtgatgttgtaataggaattgtcaacaacacagtttatgatcctttgcaacctgaattagactcattcaaggaggagttagataaatattttaagaatcatacatcaccagatgttgatttaggtgacatctctggcattaatgcttcagttgtaaacattcaaaaagaaattgaccgcctcaatgaggttgccaagaatttaaatgaatctctcatcgatctccaagaacttggaaagtatgagcagtatataaaatggccatggtacatttggctaggttttatagctggcttgattgccatagtaatggtgacaattatgctttgctgtatgaccagttgctgtagttgtctcaagggctgttgttcttgtggatcctgctgcaaatttgatgaagacgactctgagccagtgctcaaaggagtcaaattacattacacataaacgaacttatggatttgtttatgagaatcttcacaattggaactgtaactttgaagcaaggtgaaatcaaggatgctactccttcagattttgttcgcgctactgcaacgataccgatacaagcctcactccctttcggatggcttattgttggcgttgcacttcttgctgtttttcagagcgcttccaaaatcataaccctcaaaaagagatggcaactagcactctccaagggtgttcactttgtttgcaacttgctgttgttgtttgtaacagtttactcacaccttttgctcgttgctgctggccttgaagccccttttctctatctttatgctttagtctacttcttgcagagtataaactttgtaagaataataatgaggctttggctttgctggaaatgccgttccaaaaacccattactttatgatgccaactattttctttgctggcatactaattgttacgactattgtataccttacaatagtgtaacttcttcaattgtcattacttcaggtgatggcacaacaagtcctatttctgaacatgactaccagattggtggttatactgaaaaatgggaatctggagtaaaagactgtgttgtattacacagttacttcacttcagactattaccagctgtactcaactcaattgagtacagacactggtgttgaacatgttaccttcttcatctacaataaaattgttgatgagcctgaagaacatgtccaaattcacacaatcgacggttcatccggagttgttaatccagtaatggaaccaatttatgatgaaccgacgacgactactagcgtgcctttgtaagcacaagctgatgagtacgaacttatgtactcattcgtttcggaagagacaggtacgttaatagttaatagcgtacttctttttcttgctttcgtggtattcttgctagttacactagccatccttactgcgcttcgattgtgtgcgtactgctgcaatattgttaacgtgagtcttgtaaaaccttctttttacgtttactctcgtgttaaaaatctgaattcttctagagttcctgatcttctggtctaaacgaactaaatattatattagtttttctgtttggaactttaattttagccatggcagattccaacggtactattaccgttgaagagcttaaaaagctccttgaacaatggaacctagtaataggtttcctattccttacatggatttgtcttctacaatttgcctatgccaacaggaataggtttttgtatataattaagttaattttcctctggctgttatggccagtaactttagcttgttttgtgcttgctgctgtttacagaataaattggatcaccggtggaattgctatcgcaatggcttgtcttgtaggcttgatgtggctcagctacttcattgcttctttcagactgtttgcgcgtacgcgttccatgtggtcattcaatccagaaactaacattcttctcaacgtgccactccatggcactattctgaccagaccgcttctagaaagtgaactcgtaatcggagctgtgatccttcgtggacatcttcgtattgctggacaccatctaggacgctgtgacatcaaggacctgcctaaagaaatcactgttgctacatcacgaacgctttcttattacaaattgggagcttcgcagcgtgtagcaggtgactcaggttttgctgcatacagtcgctacaggattggcaactataaattaaacacagaccattccagtagcag

SEQ ID NO: 28 - DNA, 3172 bp, SARS-CoV-2
tcctctggctgttatggccagtaactttagcttgttttgtgcttgctgctgtttacagaataaattggatcaccggtggaattgctatcgcaatggcttgtcttgtaggcttgatgtggctcagctacttcattgcttctttcagactgtttgcgcgtacgcgttccatgtggtcattcaatccagaaactaacattcttctcaacgtgccactccatggcactattctgaccagaccgcttctagaaagtgaactcgtaatcggagctgtgatccttcgtggacatcttcgtattgctggacaccatctaggacgctgtgacatcaaggacctgcctaaagaaatcactgttgctacatcacgaacgctttcttattacaaattgggagcttcgcagcgtgtagcaggtgactcaggttttgctgcatacagtcgctacaggattggcaactataaattaaacacagaccattccagtagcagtgacaatattgctttgcttgtacagtaagtgacaacagatgtttcatctcgttgactttcaggttactatagcagagatattactaattattatgaggacttttaaagtttccatttggaatcttgattacatcataaacctcataattaaaaatttatctaagtcactaactgagaataaatattctcaattagatgaagagcaaccaatggagattgattaaacgaacatgaaaattattcttttcttggcactgataacactcgctacttgtgagctttatcactaccaagagtgtgttagaggtacaacagtacttttaaaagaaccttgctcttctggaacatacgagggcaattcaccatttcatcctctagctgataacaaatttgcactgacttgctttagcactcaatttgcttttgcttgtcctgacggcgtaaaacacgtctatcagttacgtgccagatcagtttcacctaaactgttcatcagacaagaggaagttcaagaactttactctccaatttttcttattgttgcggcaatagtgtttataacactttgcttcacactcaaaagaaagacagaatgattgaactttcattaattgacttctatttgtgctttttagcctttctgctattccttgttttaattatgcttattatcttttggttctcacttgaactgcaagatcataatgaaacttgtcacgcctaaacgaacatgaaatttcttgttttcttaggaatcatcacaactgtagctgcatttcaccaagaatgtagtttacagtcatgtactcaacatcaaccatatgtagttgatgacccgtgtcctattcacttctattctaaatggtatattagagtaggagctagaaaatcagcacctttaattgaattgtgcgtggatgaggctggttctaaatcacccattcagtacatcgatatcggtaattatacagtttcctgtttaccttttacaattaattgccaggaacctaaattgggtagtcttgtagtgcgttgttcgttctatgaagactttttagagtatcatgacgttcgtgttgttttagatttcatctaaacgaacaaactaaaatgtctgataatggaccccaaaatcagcgaaatgcaccccgcattacgtttggtggaccctcagattcaactggcagtaaccagaatggagaacgcagtggggcgcgatcaaaacaacgtcggccccaaggtttacccaataatactgcgtcttggttcaccgctctcactcaacatggcaaggaagaccttaaattccctcgaggacaaggcgttccaattaacaccaatagcagtccagatgaccaaattggctactaccgaagagctaccagacgaattcgtggtggtgacggtaaaatgaaagatctcagtccaagatggtatttctactacctaggaactgggccagaagctggacttccctatggtgctaacaaagacggcatcatatgggttgcaactgagggagccttgaatacaccaaaagatcacattggcacccgcaatcctgctaacaatgctgcaatcgtgctacaacttcctcaaggaacaacattgccaaaaggcttctacgcagaagggagcagaggcggcagtcaagcctcttctcgttcctcatcacgtagtcgcaacagttcaagaaattcaactccaggcagcagtaggggaacttctcctgctagaatggctggcaatggcggtgatgctgctcttgctttgctgctgcttgacagattgaaccagcttgagagcaaaatgtctggtaaaggccaacaacaacaaggccaaactgtcactaagaaatctgctgctgaggcttctaagaagcctcggcaaaaacgtactgccactaaagcatacaatgtaacacaagctttcggcagacgtggtccagaacaaacccaaggaaattttggggaccaggaactaatcagacaaggaactgattacaaacattggccgcaaattgcacaatttgcccccagcgcttcagcgttcttcggaatgtcgcgcattggcatggaagtcacaccttcgggaacgtggttgacctacacaggtgccatcaaattggatgacaaagatccaaatttcaaagatcaagtcattttgctgaataagcatattgacgcatacaaaacattcccaccaacagagcctaaaaaggacaaaaagaagaaggctgatgaaactcaagccttaccgcagagacagaagaaacagcaaactgtgactcttcttcctgctgcagatttggatgatttctccaaacaattgcaacaatccatgagcagtgctgactcaactcaggcctaaactcatgcagaccacacaaggcagatgggctatataaacgttttcgcttttccgtttacgatatatagtctactcttgtgcagaatgaattctcgtaactacatagcacaagtagatgtagttaactttaatctcacatagcaatctttaatcagtgtgtaacattagggaggacttgaaagagccaccacattttcaccgaggccacgcggagtacgatcgagtgtacagtgaacaatgctagggagagctgcctatatggaagagccctaatgtgtaaaattaattttagtagtgctatccccatgtgattttaat